European Patent Application EP 4 628 106 A1, published October 8, 2025. Title: 异二聚体及其放射性医药用途. Applicant: 核欣（苏州）医药科技有限公司. Application CN. The sequence listing filed with the application follows.

SEQUENCE LISTING (6 sequences)

SEQ ID NO: 1 - protein, 5 aa, Artificial Sequence
  REGION 1..5: note = circular
  SITE 4: note = D-phenylalanine
RGDFK

SEQ ID NO: 2 - protein, 5 aa, Artificial Sequence
  REGION 1..5: note = circular
  SITE 4: note = D-Tyrosine
RGDYK

SEQ ID NO: 3 - protein, 6 aa, Artificial Sequence
  REGION 1..6: note = circular
KYNGRT

SEQ ID NO: 4 - protein, 6 aa, Artificial Sequence
  REGION 1..6: note = circular
  SITE 4: note = MeGly
KGNXRG

SEQ ID NO: 5 - protein, 5 aa, Artificial Sequence
  REGION 1..5: note = circular
KNGRE

SEQ ID NO: 6 - protein, 6 aa, Artificial Sequence
  REGION 1..6: note = circular
  SITE 4: note = MeGly
KYNXRT